European Patent Specification EP 3 891 176 B1, published June 5, 2024. Title: GLP-1 and Neurotensin receptor co-agonist. Applicant: Københavns Universitet. The sequence listing filed with the application follows.

SEQUENCE LISTING (70 sequences)

SEQ ID NO: 1 - protein, 9 aa, Homo sapiens
  GLP-1 (7-15 aa)
HAEGTFTSD

SEQ ID NO: 2 - protein, 30 aa, Homo sapiens
  GLP-1 (7-36)
HAEGTFTSDVSSYLEGQAAKEFIAWLVKGR

SEQ ID NO: 3 - protein, 29 aa, Homo sapiens
  GLP-1 (7-35)
HAEGTFTSDVSSYLEGQAAKEFIAWLVKG

SEQ ID NO: 4 - protein, 28 aa, Homo sapiens
  GLP-1 (7-34)
HAEGTFTSDVSSYLEGQAAKEFIAWLVK

SEQ ID NO: 5 - protein, 27 aa, Homo sapiens
  GLP-1 (7-33)
HAEGTFTSDVSSYLEGQAAKEFIAWLV

SEQ ID NO: 6 - protein, 26 aa, Homo sapiens
  GLP-1 (7-32)
HAEGTFTSDVSSYLEGQAAKEFIAWL

SEQ ID NO: 7 - protein, 25 aa, Homo sapiens
  GLP-1 (7-31)
HAEGTFTSDVSSYLEGQAAKEFIAW

SEQ ID NO: 8 - protein, 24 aa, Homo sapiens
  GLP-1 (7-30)
HAEGTFTSDVSSYLEGQAAKEFIA

SEQ ID NO: 9 - protein, 23 aa, Homo sapiens
  GLP-1 (7-29)
HAEGTFTSDVSSYLEGQAAKEFI

SEQ ID NO: 10 - protein, 22 aa, Homo sapiens
  GLP-1 (7-28)
HAEGTFTSDVSSYLEGQAAKEF

SEQ ID NO: 11 - protein, 21 aa, Homo sapiens
  GLP-1 (7-27)
HAEGTFTSDVSSYLEGQAAKE

SEQ ID NO: 12 - protein, 20 aa, Homo sapiens
  GLP-1 (7-26)
HAEGTFTSDVSSYLEGQAAK

SEQ ID NO: 13 - protein, 19 aa, Homo sapiens
  GLP-1 (7-25)
HAEGTFTSDVSSYLEGQAA

SEQ ID NO: 14 - protein, 18 aa, Homo sapiens
  GLP-1 (7-24)
HAEGTFTSDVSSYLEGQA

SEQ ID NO: 15 - protein, 17 aa, Homo sapiens
  GLP-1 (7-23)
HAEGTFTSDVSSYLEGQ

SEQ ID NO: 16 - protein, 16 aa, Homo sapiens
  GLP-1 (7-22)
HAEGTFTSDVSSYLEG

SEQ ID NO: 17 - protein, 15 aa, Homo sapiens
  GLP-1 (7-21)
HAEGTFTSDVSSYLE

SEQ ID NO: 18 - protein, 14 aa, Homo sapiens
  GLP-1 (7-20)
HAEGTFTSDVSSYL

SEQ ID NO: 19 - protein, 13 aa, Homo sapiens
  GLP-1 (7-19)
HAEGTFTSDVSSY

SEQ ID NO: 20 - protein, 12 aa, Homo sapiens
  GLP-1 (7-18)
HAEGTFTSDVSS

SEQ ID NO: 21 - protein, 11 aa, Homo sapiens
  GLP-1 (7-17)
HAEGTFTSDVS

SEQ ID NO: 22 - protein, 10 aa, Homo sapiens
  GLP-1 (7-16)
HAEGTFTSDV

SEQ ID NO: 23 - protein, 8 aa, Homo sapiens
  GLP-1 (7-14)
HAEGTFTS

SEQ ID NO: 24 - protein, 13 aa, Homo sapiens
  Neurotensin (NT) (1-13)
QLYENKPRRPYIL

SEQ ID NO: 25 - protein, 12 aa, Homo sapiens
  NT (2-13)
LYENKPRRPYIL

SEQ ID NO: 26 - protein, 11 aa, Homo sapiens
  NT (3-13)
YENKPRRPYIL

SEQ ID NO: 27 - protein, 10 aa, Homo sapiens
  NT (4-13)
ENKPRRPYIL

SEQ ID NO: 28 - protein, 9 aa, Homo sapiens
  NT (5-13)
NKPRRPYIL

SEQ ID NO: 29 - protein, 8 aa, Homo sapiens
  NT (6-13)
KPRRPYIL

SEQ ID NO: 30 - protein, 7 aa, Homo sapiens
  NT (7-13)
PRRPYIL

SEQ ID NO: 31 - protein, 6 aa, Homo sapiens
  NT (8-13)
RRPYIL

SEQ ID NO: 32 - protein, 43 aa, Artificial Sequence
  GLP-1 (7-36)/NT (1-13)
HAEGTFTSDVSSYLEGQAAKEFIAWLVKGRQLYENKPRRPYIL

SEQ ID NO: 33 - protein, 52 aa, Artificial Sequence
  Exendin 4/NT (1-13)
HGEGTFTSDLSKQMEEEAVRLFIEWLKNGGPSSGAPPPSQLYENKPRRPYIL

SEQ ID NO: 34 - protein, 39 aa, Homo sapiens
  Exendin 4
HGEGTFTSDLSKQMEEEAVRLFIEWLKNGGPSSGAPPPS

SEQ ID NO: 35 - protein, 34 aa, Homo sapiens
  GLP-2
HADGSFSDEMNTILDNLAARDFINWLIQTKITDR

SEQ ID NO: 36 - protein, 29 aa, Homo sapiens
  Glucagon
HSQGTFTSDYSKYLDSRRAQDFVQWLMNT

SEQ ID NO: 37 - protein, 28 aa, Homo sapiens
  VIP
HSDAVFTDNYTRLRKQMAVKKYLNSILN

SEQ ID NO: 38 - protein, 33 aa, Homo sapiens
  Secretin
HSDGTFTSELSRLREGARLQRLLQGLVGKRSEQ

SEQ ID NO: 39 - protein, 38 aa, Homo sapiens
  PACAP-38
HSDGIFTDSYSRYRKQMAVKKYLAAVLGKRYKQRVKNK

SEQ ID NO: 40 - protein, 10 aa, Homo sapiens
  NKA
HKTDSFVGLM

SEQ ID NO: 41 - protein, 34 aa, Homo sapiens
  PYY
IKPEAPREDASPEELNRYYASLRHYLNLVTRQRY

SEQ ID NO: 42 - protein, 37 aa, Homo sapiens [sequence omitted]

SEQ ID NO: 43 - protein, 44 aa, Artificial Sequence
  GLP(7-37)/NT(1-13)
HAEGTFTSDVSSYLEGQAAKEFIAWLVKGRGQLYENKPRRPYIL

SEQ ID NO: 44 - protein, 31 aa, Homo sapiens
  GLP-1 (7-37)
HAEGTFTSDVSSYLEGQAAKEFIAWLVKGRG

SEQ ID NO: 45 - protein, 42 aa, Artificial Sequence
  GLP-1 (7-36)/NT (2-13)
HAEGTFTSDVSSYLEGQAAKEFIAWLVKGRLYENKPRRPYIL

SEQ ID NO: 46 - protein, 43 aa, Artificial Sequence
  GLP-1 (7-37)/NT(2-13)
HAEGTFTSDVSSYLEGQAAKEFIAWLVKGRGLYENKPRRPYIL

SEQ ID NO: 47 - protein, 4 aa, Artificial Sequence
  Synthetic sequence
KKGG

SEQ ID NO: 48 - protein, 9 aa, Homo sapiens
  VARIANT 1: L-histidine, D-histidine, desamino-histidine, 2-amino-histidine, β hydroxy-histidine, homohistidine, Nα-acetyl-histidine, α-fluoromethyl-histidine, α-methyl-histidine, 3-pyridylalanine, 2-pyridylalanine or 4 pyridylalanine
  VARIANT 2: A, G, V, L, I, K, S, aminoisobutyric acid (Aib), (1-aminocyclopro pyl) carboxylic acid, (1 aminocyclobutyl) carboxylic acid, (1-ami nocyclopentyl) carboxylic acid, (1 aminocyclohexyl) carboxylic ac id, (1-aminocycloheptyl) carboxylic acid, or (1-aminocycloocty
  VARIANT 3: E, D or Q
  VARIANT 4: G or A
  VARIANT 5: T, V, S or I
  VARIANT 6: F or Y
  VARIANT 7: T or S
  VARIANT 8: S, V or D
  VARIANT 9: S, D, E or is not present
XXXXXXXXX

SEQ ID NO: 49 - protein, 6 aa, Homo sapiens
  VARIANT 1: R or K
  VARIANT 2: R or K
  VARIANT 4: Y, S, C or T
XXPXIL

SEQ ID NO: 50 - protein, 7 aa, Homo sapiens
  VARIANT 2: R or K
  VARIANT 3: R or K
  VARIANT 5: Y, S, C or T
PXXPXIL

SEQ ID NO: 51 - protein, 8 aa, Homo sapiens
  VARIANT 3: R or K
  VARIANT 4: R or K
  VARIANT 6: Y, S, C or T
KPXXPXIL

SEQ ID NO: 52 - protein, 9 aa, Homo sapiens
  VARIANT 4: R or K
  VARIANT 5: R or K
  VARIANT 7: Y, S, C or T
NKPXXPXIL

SEQ ID NO: 53 - protein, 10 aa, Homo sapiens
  VARIANT 5: R or K
  VARIANT 6: R or K
  VARIANT 8: Y, S, C or T
ENKPXXPXIL

SEQ ID NO: 54 - protein, 11 aa, Homo sapiens
  VARIANT 6: R or K
  VARIANT 7: R or K
  VARIANT 9: Y, S, C or T
YENKPXXPXIL

SEQ ID NO: 55 - protein, 12 aa, Homo sapiens
  VARIANT 7: R or K
  VARIANT 8: R or K
  VARIANT 10: Y, S, C or T
LYENKPXXPXIL

SEQ ID NO: 56 - protein, 13 aa, Homo sapiens
  VARIANT 8: R or K
  VARIANT 9: R or K
  VARIANT 11: Y, S, C or T
QLYENKPXXPXIL

SEQ ID NO: 57 - protein, 15 aa, Artificial Sequence
  GLP-1 (7-15)/NT (1-6)
HAEGTFTSDRRPYIL

SEQ ID NO: 58 - protein, 19 aa, Artificial Sequence
  GLP-1 (7-15)/KKGG Linker/NT (1-6)
HAEGTFTSDKKGGRRPYIL

SEQ ID NO: 59 - protein, 23 aa, Artificial Sequence
  GLP-1 (7-19)/NT (1-10)
HAEGTFTSDVSSYENKPRRPYIL

SEQ ID NO: 60 - protein, 27 aa, Artificial Sequence
  GLP-1 (7-19)/KKGG Linker/NT (1-10)
HAEGTFTSDVSSYKKGGENKPRRPYIL

SEQ ID NO: 61 - protein, 30 aa, Artificial Sequence
  GLP-1 (7-23)/NT (1-13)
HAEGTFTSDVSSYLEGQELYENKPRRPYIL

SEQ ID NO: 62 - protein, 34 aa, Artificial Sequence
  GLP-1 (7-23)/KKGG Linker/NT (1-13)
HAEGTFTSDVSSYLEGQKKGGELYENKPRRPYIL

SEQ ID NO: 63 - protein, 33 aa, Artificial Sequence
  GLP-1 (7-26)/NT (1-13)
HAEGTFTSDVSSYLEGQAAKELYENKPRRPYIL

SEQ ID NO: 64 - protein, 37 aa, Artificial Sequence
  GLP-1 (7-26)/KKGG Linker/NT (1-13)
HAEGTFTSDVSSYLEGQAAKKKGGELYENKPRRPYIL

SEQ ID NO: 65 - protein, 43 aa, Artificial Sequence
  GLP-1 (7-35)/PEGylated NT (1-13)
  MOD_RES 36: PEGylation
HAEGTFTSDVSSYLEGQAAKEFIAWLVKGRELYENKPRRPYIL

SEQ ID NO: 66 - protein, 47 aa, Artificial Sequence
  GLP-1 (7-35)/KKGG linker/PEGylated NT (1-13)
  MOD_RES 40: PEGylation
HAEGTFTSDVSSYLEGQAAKEFIAWLVKGRKKGGELYENKPRRPYIL

SEQ ID NO: 67 - protein, 43 aa, Artificial Sequence; identical to SEQ ID NO: 65
  GLP-1 (7-35)/NT (1-13)

SEQ ID NO: 68 - protein, 47 aa, Artificial Sequence; identical to SEQ ID NO: 66
  GLP-1 (7-35)/KKGG linker/NT (1-13)

SEQ ID NO: 69 - protein, 13 aa, Homo sapiens
  NT (1-13)
ELYENKPRRPYIL

SEQ ID NO: 70 - protein, 13 aa, Homo sapiens
  PEGylated NT (1-13)
  MOD_RES 6: PEGylation
ELYENKPRRPYIL